European Patent Application EP 4 235 179 A2, published August 30, 2023. Title: DETECTION, QUANTIFICATION OR ISOLATION OF TUMOR CELLS. Applicant: Université Libre de Bruxelles. Application EP. The sequence listing filed with the application follows.

SEQUENCE LISTING (3 sequences)

SEQ ID NO: 1 - DNA, 900 bp, Homo sapiens
  source 1..900: mol_type = other DNA
atggggacaaaggcgcaagtcgagaggaaactgttgtgcctcttcatattggcgatcctgttgtgctccctggcattgggcagtgttacagtgcactcttctgaacctgaagtcagaattcctgagaataatcctgtgaagttgtcctgtgcctactcgggcttttcttctccccgtgtggagtggaagtttgaccaaggagacaccaccagactcgtttgctataataacaagatcacagcttcctatgaggaccgggtgaccttcttgccaactggtatcaccttcaagtccgtgacacgggaagacactgggacatacacttgtatggtctctgaggaaggcggcaacagctatggggaggtcaaggtcaagctcatcgtgcttgtgcctccatccaagcctacagttaacatcccctcctctgccaccattgggaaccgggcagtgctgacatgctcagaacaagatggttccccaccttctgaatacacctggttcaaagatgggatagtgatgcctacgaatcccaaaagcacccgtgccttcagcaactcttcctatgtcctgaatcccacaacaggagagctggtctttgatcccctgtcagcctctgatactggagaatacagctgtgaggcacggaatgggtatgggacacccatgacttcaaatgctgtgcgcatggaagctgtggagcggaatgtgggggtcatcgtggcagccgtccttgtaaccctgattctcctgggaatcttggtttttggcatctggtttgcctatagccgaggccactttgacagaacaaagaaagggacttcgagtaagaaggtgatttacagccagcctagtgcccgaagtgaaggagaattcaaacagacctcgtcattcctggtgtga

SEQ ID NO: 2 - protein, 299 aa, Homo sapiens
MGTKAQVERKLLCLFILAILLCSLALGSVTVHSSEPEVRIPENNPVKLSCAYSGFSSPRVEWKFDQGDTTRLVCYNNKITASYEDRVTFLPTGITFKSVTREDTGTYTCMVSEEGGNSYGEVKVKLIVLVPPSKPTVNIPSSATIGNRAVLTCSEQDGSPPSEYTWFKDGIVMPTNPKSTRAFSNSSYVLNPTTGELVFDPLSASDTGEYSCEARNGYGTPMTSNAVRMEAVERNVGVIVAAVLVTLILLGILVFGIWFAYSRGHFDRTKKGTSSKKVIYSQPSARSEGEFKQTSSFLV

SEQ ID NO: 3 - protein, 250 aa, Homo sapiens
MGTKAQVERKLLCLFILAILLCSLALGSVTVHSSEPEVRIPENNPVKLSCAYSGFSSPRVEWKFDQGDTTRLVCYNNKITVPPSKPTVNIPSSATIGNRAVLTCSEQDGSPPSEYTWFKDGIVMPTNPKSTRAFSNSSYVLNPTTGELVFDPLSASDTGEYSCEARNGYGTPMTSNAVRMEAVERNVGVIVAAVLVTLILLGILVFGIWFAYSRGHFDRTKKGTSSKKVIYSQPSARSEGEFKQTSSFLV